European Patent Specification EP 3 139 960 B1, published January 17, 2024. Title: Liquid formulation comprising GM-CSF neutralizing compound. Applicant: Takeda. The sequence listing filed with the application follows.

SEQUENCE LISTING (60 sequences)

SEQ ID NO: 1 - protein, 10 aa, artificial sequence
  CDR-H3 7A-701
SGLIANHMTP

SEQ ID NO: 2 - protein, 10 aa, artificial sequence
  CDR-H3 7B1-502
TTLISVYFDY

SEQ ID NO: 3 - protein, 10 aa, artificial sequence
  CDR-H3 L38-A1
SGLIFDYWLD

SEQ ID NO: 4 - protein, 10 aa, artificial sequence
  CDR-H3 L38-A12
SGLIIDALSP

SEQ ID NO: 5 - protein, 10 aa, artificial sequence
  CDR-H3 L38-G7
TSLMSIYFDY

SEQ ID NO: 6 - protein, 10 aa, artificial sequence
  CDR-H3 L39-D11
SGLLFLYFDY

SEQ ID NO: 7 - protein, 10 aa, artificial sequence
  CDR-H3 E1-37-E7
SGLINLGMHP

SEQ ID NO: 8 - protein, 10 aa, artificial sequence
  CDR-H3 M1_3-82
SGLIFDALRD

SEQ ID NO: 9 - protein, 10 aa, artificial sequence
  CDR-H3 Ln4p-23
SGLIFDKLTS

SEQ ID NO: 10 - protein, 10 aa, artificial sequence
  CDR-H3 Ln4p-28
SGLINLHFDT

SEQ ID NO: 11 - protein, 10 aa, artificial sequence
  CDR-H3 Ln4p-50
STHFSAYFDY

SEQ ID NO: 12 - protein, 10 aa, artificial sequence
  CDR-H3 Ln4p-65
SGLIMDKLDN

SEQ ID NO: 13 - protein, 10 aa, artificial sequence
  CDR-H3 Ln4p-90
SGLIIDNLNP

SEQ ID NO: 14 - protein, 5 aa, artificial sequence
  CDR-H1 7B1-502
DYLLH

SEQ ID NO: 15 - protein, 17 aa, artificial sequence
  CDR-H2 7B1-502
WLNPYSGDTNYAQKFQG

SEQ ID NO: 16 - protein, 11 aa, artificial sequence
  CDR-L1 5-306
RASQNIRNILN

SEQ ID NO: 17 - protein, 7 aa, artificial sequence
  CDR-L2 5-306
AASNLQS

SEQ ID NO: 18 - protein, 9 aa, artificial sequence
  CDR-L3 5-306
QQSYSMPRT

SEQ ID NO: 19 - protein, 107 aa, artificial sequence
  VL 5-306* L-version
DIQMTQSPSSVSASVGDRVTIACRASQNIRNILNWYQQRPGKAPQLLIYAASNLQSGVPSRFSGSGSGTDFTLTINSLQPEDFATYYCQQSYSMPRTFGGGTKLEIK

SEQ ID NO: 20 - protein, 119 aa, artificial sequence
  VH with CDR-H3 = 7A-701
EVQLLESGAEVKKPGASVKVSCKAFGYPFTDYLLHWVRQAPGQGLEWVGWLNPYSGDTNYAQKFQGRVTMTRDTSISTAYMELSRLRSDDTAVYYCTRSGLIANHMTPWGQGTMVTVSS

SEQ ID NO: 21 - protein, 119 aa, artificial sequence
  VH with CDR-H3 = 7B1-502*
QVQLVQSGAEVKKPGASVKVSCKAFGYPFTDYLLHWVRQAPGQGLEWVGWLNPYSGDTNYAQKFQGRVTMTRDTSISTAYMELSRLRSDDTAVYYCTRTTLISVYFDYWGQGTMVTVSS

SEQ ID NO: 22 - protein, 119 aa, artificial sequence
  VH with CDR-H3 = 3077*
QVQLVQSGAEVKKPGASVKVSCKAFGYPFTDYLLHWVRQAPGQGLEWVGWLNPYSGDTNYAQKFQGRVTMTRDTSISTAYMELSRLRSDDTAVYYCTRSGLIAVYFDYWGQGTMVTVSS

SEQ ID NO: 23 - protein, 119 aa, artificial sequence
  VH with CDR-H3 = L38-A1
EVQLLESGAEVKKPGASVKVSCKAFGYPFTDYLLHWVRQAPGQGLEWVGWLNPYSGDTNYAQKFQGRVTMTRDTSISTAYMELSRLRSDDTAVYYCARSGLIFDYWLDWGQGTMVTVSS

SEQ ID NO: 24 - protein, 119 aa, artificial sequence
  VH with CDR-H3 = L38-A12
EVQLLESGAEVKKPGASVKVSCKAFGYPFTDYLLHWVRQAPGQGLEWVGWLNPYSGDTNYAQKFQGRVTMTRDTSISTAYMELSRLRSDDTAVYYCARSGLIIDALSPWGQGTMVTVSS

SEQ ID NO: 25 - protein, 119 aa, artificial sequence
  VH with CDR-H3 = L38-G7
EVQLLESGAEVKKPGASVKVSCKAFGYPFTDYLLHWVRQAPGQGLEWVGWLNPYSGDTNYAQKFQGRVTMTRDTSISTAYMELSRLRSDDTAVYYCTRTSLMSIYFDYWGQGTMVTVSS

SEQ ID NO: 26 - protein, 119 aa, artificial sequence
  VH with CDR-H3 = L39-D11
EVQLLESGAEVKKPGASVKVSCKAFGYPFTDYLLHWVRQAPGQGLEWVGWLNPYSGDTNYAQKFQGRVTMTRDTSISTAYMELSRLRSDDTAVYYCTRSGLLFLYFDYWGQGTMVTVSS

SEQ ID NO: 27 - protein, 119 aa, artificial sequence
  VH with CDR-H3 = E1-37-E7
EVQLLESGAEVKKPGASVKVSCKAFGYPFTDYLLHWVRQAPGQGLEWVGWLNPYSGDTNYAQKFQGRVTMTRDTSISTAYMELSRLRSDDTAVYYCARSGLINLGMHPWGQGTMVTVSS

SEQ ID NO: 28 - protein, 119 aa, artificial sequence
  VH with CDR-H3 = M1_3-82
EVQLLESGAEVKKPGASVKVSCKAFGYPFTDYLLHWVRQAPGQGLEWVGWLNPYSGDTNYAQKFQGRVTMTRDTSISTAYMELSRLRSDDTAVYYCARSGLIFDALRDWGQGTMVTVSS

SEQ ID NO: 29 - protein, 119 aa, artificial sequence
  VH with CDR-H3 = Ln4p-23
EVQLLESGAEVKKPGASVKVSCKAFGYPFTDYLLHWVRQAPGQGLEWVGWLNPYSGDTNYAQKFQGRVTMTRDTSISTAYMELSRLRSDDTAVYYCARSGLIFDKLTSWGQGTMVTVSS

SEQ ID NO: 30 - protein, 119 aa, artificial sequence
  VH with CDR-H3 = Ln4p-28
EVQLLESGAEVKKPGASVKVSCKAFGYPFTDYLLHWVRQAPGQGLEWVGWLNPYSGDTNYAQKFQGRVTMTRDTSISTAYMELSRLRSDDTAVYYCARSGLINLHFDTWGQGTMVTVSS

SEQ ID NO: 31 - protein, 119 aa, artificial sequence
  VH with CDR-H3 = Ln4p-50
EVQLLESGAEVKKPGASVKVSCKAFGYPFTDYLLHWVRQAPGQGLEWVGWLNPYSGDTNYAQKFQGRVTMTRDTSISTAYMELSRLRSDDTAVYYCTRSTHFSAYFDYWGQGTMVTVSS

SEQ ID NO: 32 - protein, 119 aa, artificial sequence
  VH with CDR-H3 = Ln4p-65
EVQLLESGAEVKKPGASVKVSCKAFGYPFTDYLLHWVRQAPGQGLEWVGWLNPYSGDTNYAQKFQGRVTMTRDTSISTAYMELSRLRSDDTAVYYCARSGLIMDKLDNWGQGTMVTVSS

SEQ ID NO: 33 - protein, 119 aa, artificial sequence
  VH with CDR-H3 = Ln4p-90
EVQLLESGAEVKKPGASVKVSCKAFGYPFTDYLLHWVRQAPGQGLEWVGWLNPYSGDTNYAQKFQGRVTMTRDTSISTAYMELSRLRSDDTAVYYCARSGLIIDNLNPWGQGTMVTVSS

SEQ ID NO: 34 - protein, 214 aa, artificial sequence
  Light Chain 5-306* L-version
DIQMTQSPSSVSASVGDRVTIACRASQNIRNILNWYQQRPGKAPQLLIYAASNLQSGVPSRFSGSGSGTDFTLTINSLQPEDFATYYCQQSYSMPRTFGGGTKLEIKRTVAAPSVFIFPPSDEQLKSGTASVVCLLNNFYPREAKVQWKVDNALQSGNSQESVTEQDSKDSTYSLSSTLTLSKADYEKHKVYACEVTHQGLSSPVTKSFNRGEC

SEQ ID NO: 35 - protein, 449 aa, artificial sequence
  Heavy Chain with CDR-H3 = 7B1-502*
QVQLVQSGAEVKKPGASVKVSCKAFGYPFTDYLLHWVRQAPGQGLEWVGWLNPYSGDTNYAQKFQGRVTMTRDTSISTAYMELSRLRSDDTAVYYCTRTTLISVYFDYWGQGTMVTVSSASTKGPSVFPLAPSSKSTSGGTAALGCLVKDYFPEPVTVSWNSGALTSGVHTFPAVLQSSGLYSLSSVVTVPSSSLGTQTYICNVNHKPSNTKVDKKVEPKSCDKTHTCPPCPAPELLGGPSVFLFPPKPKDTLMISRTPEVTCVVVDVSHEDPEVKFNWYVDGVEVHNAKTKPREEQYNSTYRVVSVLTVLHQDWLNGKEYKCKVSNKALPAPIEKTISKAKGQPREPQVYTLPPSRDELTKNQVSLTCLVKGFYPSDIAVEWESNGQPENNYKTTPPVLDSDGSFFLYSKLTVDKSRWQQGNVFSCSVMHEALHNHYTQKSLSLSPGK

SEQ ID NO: 36 - protein, 449 aa, artificial sequence
  Heavy Chain with CDR-H3 =7A-701*
QVQLVQSGAEVKKPGASVKVSCKAFGYPFTDYLLHWVRQAPGQGLEWVGWLNPYSGDTNYAQKFQGRVTMTRDTSISTAYMELSRLRSDDTAVYYCTRSGLIANHMTPWGQGTMVTVSSASTKGPSVFPLAPSSKSTSGGTAALGCLVKDYFPEPVTVSWNSGALTSGVHTFPAVLQSSGLYSLSSVVTVPSSSLGTQTYICNVNHKPSNTKVDKKVEPKSCDKTHTCPPCPAPELLGGPSVFLFPPKPKDTLMISRTPEVTCVVVDVSHEDPEVKFNWYVDGVEVHNAKTKPREEQYNSTYRVVSVLTVLHQDWLNGKEYKCKVSNKALPAPIEKTISKAKGQPREPQVYTLPPSRDELTKNQVSLTCLVKGFYPSDIAVEWESNGQPENNYKTTPPVLDSDGSFFLYSKLTVDKSRWQQGNVFSCSVMHEALHNHYTQKSLSLSPGK

SEQ ID NO: 37 - protein, 449 aa, artificial sequence
  Heavy Chain with CDR-H3 = L38-A1*
QVQLVQSGAEVKKPGASVKVSCKAFGYPFTDYLLHWVRQAPGQGLEWVGWLNPYSGDTNYAQKFQGRVTMTRDTSISTAYMELSRLRSDDTAVYYCARSGLIFDYWLDWGQGTMVTVSSASTKGPSVFPLAPSSKSTSGGTAALGCLVKDYFPEPVTVSWNSGALTSGVHTFPAVLQSSGLYSLSSVVTVPSSSLGTQTYICNVNHKPSNTKVDKKVEPKSCDKTHTCPPCPAPELLGGPSVFLFPPKPKDTLMISRTPEVTCVVVDVSHEDPEVKFNWYVDGVEVHNAKTKPREEQYNSTYRVVSVLTVLHQDWLNGKEYKCKVSNKALPAPIEKTISKAKGQPREPQVYTLPPSRDELTKNQVSLTCLVKGFYPSDIAVEWESNGQPENNYKTTPPVLDSDGSFFLYSKLTVDKSRWQQGNVFSCSVMHEALHNHYTQKSLSLSPGK

SEQ ID NO: 38 - protein, 449 aa, artificial sequence
  Heavy Chain with CDR-H3 = L38-A12*
QVQLVQSGAEVKKPGASVKVSCKAFGYPFTDYLLHWVRQAPGQGLEWVGWLNPYSGDTNYAQKFQGRVTMTRDTSISTAYMELSRLRSDDTAVYYCARSGLIIDALSPWGQGTMVTVSSASTKGPSVFPLAPSSKSTSGGTAALGCLVKDYFPEPVTVSWNSGALTSGVHTFPAVLQSSGLYSLSSVVTVPSSSLGTQTYICNVNHKPSNTKVDKKVEPKSCDKTHTCPPCPAPELLGGPSVFLFPPKPKDTLMISRTPEVTCVVVDVSHEDPEVKFNWYVDGVEVHNAKTKPREEQYNSTYRVVSVLTVLHQDWLNGKEYKCKVSNKALPAPIEKTISKAKGQPREPQVYTLPPSRDELTKNQVSLTCLVKGFYPSDIAVEWESNGQPENNYKTTPPVLDSDGSFFLYSKLTVDKSRWQQGNVFSCSVMHEALHNHYTQKSLSLSPGK

SEQ ID NO: 39 - protein, 449 aa, artificial sequence
  Heavy Chain with CDR-H3 = L38-G7*
QVQLVQSGAEVKKPGASVKVSCKAFGYPFTDYLLHWVRQAPGQGLEWVGWLNPYSGDTNYAQKFQGRVTMTRDTSISTAYMELSRLRSDDTAVYYCTRTSLMSIYFDYWGQGTMVTVSSASTKGPSVFPLAPSSKSTSGGTAALGCLVKDYFPEPVTVSWNSGALTSGVHTFPAVLQSSGLYSLSSVVTVPSSSLGTQTYICNVNHKPSNTKVDKKVEPKSCDKTHTCPPCPAPELLGGPSVFLFPPKPKDTLMISRTPEVTCVVVDVSHEDPEVKFNWYVDGVEVHNAKTKPREEQYNSTYRVVSVLTVLHQDWLNGKEYKCKVSNKALPAPIEKTISKAKGQPREPQVYTLPPSRDELTKNQVSLTCLVKGFYPSDIAVEWESNGQPENNYKTTPPVLDSDGSFFLYSKLTVDKSRWQQGNVFSCSVMHEALHNHYTQKSLSLSPGK

SEQ ID NO: 40 - protein, 449 aa, artificial sequence
  Heavy Chain with CDR-H3 = L39-D11*
QVQLVQSGAEVKKPGASVKVSCKAFGYPFTDYLLHWVRQAPGQGLEWVGWLNPYSGDTNYAQKFQGRVTMTRDTSISTAYMELSRLRSDDTAVYYCTRSGLLFLYFDYWGQGTMVTVSSASTKGPSVFPLAPSSKSTSGGTAALGCLVKDYFPEPVTVSWNSGALTSGVHTFPAVLQSSGLYSLSSVVTVPSSSLGTQTYICNVNHKPSNTKVDKKVEPKSCDKTHTCPPCPAPELLGGPSVFLFPPKPKDTLMISRTPEVTCVVVDVSHEDPEVKFNWYVDGVEVHNAKTKPREEQYNSTYRVVSVLTVLHQDWLNGKEYKCKVSNKALPAPIEKTISKAKGQPREPQVYTLPPSRDELTKNQVSLTCLVKGFYPSDIAVEWESNGQPENNYKTTPPVLDSDGSFFLYSKLTVDKSRWQQGNVFSCSVMHEALHNHYTQKSLSLSPGK

SEQ ID NO: 41 - protein, 449 aa, artificial sequence
  Heavy Chain with CDR-H3 = E1-37-E7*
QVQLVQSGAEVKKPGASVKVSCKAFGYPFTDYLLHWVRQAPGQGLEWVGWLNPYSGDTNYAQKFQGRVTMTRDTSISTAYMELSRLRSDDTAVYYCARSGLINLGMHPWGQGTMVTVSSASTKGPSVFPLAPSSKSTSGGTAALGCLVKDYFPEPVTVSWNSGALTSGVHTFPAVLQSSGLYSLSSVVTVPSSSLGTQTYICNVNHKPSNTKVDKKVEPKSCDKTHTCPPCPAPELLGGPSVFLFPPKPKDTLMISRTPEVTCVVVDVSHEDPEVKFNWYVDGVEVHNAKTKPREEQYNSTYRVVSVLTVLHQDWLNGKEYKCKVSNKALPAPIEKTISKAKGQPREPQVYTLPPSRDELTKNQVSLTCLVKGFYPSDIAVEWESNGQPENNYKTTPPVLDSDGSFFLYSKLTVDKSRWQQGNVFSCSVMHEALHNHYTQKSLSLSPGK

SEQ ID NO: 42 - protein, 449 aa, artificial sequence
  Heavy Chain with CDR-H3 = M1_3-82*
QVQLVQSGAEVKKPGASVKVSCKAFGYPFTDYLLHWVRQAPGQGLEWVGWLNPYSGDTNYAQKFQGRVTMTRDTSISTAYMELSRLRSDDTAVYYCARSGLIFDALRDWGQGTMVTVSSASTKGPSVFPLAPSSKSTSGGTAALGCLVKDYFPEPVTVSWNSGALTSGVHTFPAVLQSSGLYSLSSVVTVPSSSLGTQTYICNVNHKPSNTKVDKKVEPKSCDKTHTCPPCPAPELLGGPSVFLFPPKPKDTLMISRTPEVTCVVVDVSHEDPEVKFNWYVDGVEVHNAKTKPREEQYNSTYRVVSVLTVLHQDWLNGKEYKCKVSNKALPAPIEKTISKAKGQPREPQVYTLPPSRDELTKNQVSLTCLVKGFYPSDIAVEWESNGQPENNYKTTPPVLDSDGSFFLYSKLTVDKSRWQQGNVFSCSVMHEALHNHYTQKSLSLSPGK

SEQ ID NO: 43 - protein, 449 aa, artificial sequence
  Heavy Chain with CDR-H3 = Ln4p-23*
QVQLVQSGAEVKKPGASVKVSCKAFGYPFTDYLLHWVRQAPGQGLEWVGWLNPYSGDTNYAQKFQGRVTMTRDTSISTAYMELSRLRSDDTAVYYCARSGLIFDKLTSWGQGTMVTVSSASTKGPSVFPLAPSSKSTSGGTAALGCLVKDYFPEPVTVSWNSGALTSGVHTFPAVLQSSGLYSLSSVVTVPSSSLGTQTYICNVNHKPSNTKVDKKVEPKSCDKTHTCPPCPAPELLGGPSVFLFPPKPKDTLMISRTPEVTCVVVDVSHEDPEVKFNWYVDGVEVHNAKTKPREEQYNSTYRVVSVLTVLHQDWLNGKEYKCKVSNKALPAPIEKTISKAKGQPREPQVYTLPPSRDELTKNQVSLTCLVKGFYPSDIAVEWESNGQPENNYKTTPPVLDSDGSFFLYSKLTVDKSRWQQGNVFSCSVMHEALHNHYTQKSLSLSPGK

SEQ ID NO: 44 - protein, 449 aa, artificial sequence
  Heavy Chain with CDR-H3 = Ln4p-28*
QVQLVQSGAEVKKPGASVKVSCKAFGYPFTDYLLHWVRQAPGQGLEWVGWLNPYSGDTNYAQKFQGRVTMTRDTSISTAYMELSRLRSDDTAVYYCARSGLINLHFDTWGQGTMVTVSSASTKGPSVFPLAPSSKSTSGGTAALGCLVKDYFPEPVTVSWNSGALTSGVHTFPAVLQSSGLYSLSSVVTVPSSSLGTQTYICNVNHKPSNTKVDKKVEPKSCDKTHTCPPCPAPELLGGPSVFLFPPKPKDTLMISRTPEVTCVVVDVSHEDPEVKFNWYVDGVEVHNAKTKPREEQYNSTYRVVSVLTVLHQDWLNGKEYKCKVSNKALPAPIEKTISKAKGQPREPQVYTLPPSRDELTKNQVSLTCLVKGFYPSDIAVEWESNGQPENNYKTTPPVLDSDGSFFLYSKLTVDKSRWQQGNVFSCSVMHEALHNHYTQKSLSLSPGK

SEQ ID NO: 45 - protein, 449 aa, artificial sequence
  Heavy Chain with CDR-H3 = Ln4p-50*
QVQLVQSGAEVKKPGASVKVSCKAFGYPFTDYLLHWVRQAPGQGLEWVGWLNPYSGDTNYAQKFQGRVTMTRDTSISTAYMELSRLRSDDTAVYYCTRSTHFSAYFDYWGQGTMVTVSSASTKGPSVFPLAPSSKSTSGGTAALGCLVKDYFPEPVTVSWNSGALTSGVHTFPAVLQSSGLYSLSSVVTVPSSSLGTQTYICNVNHKPSNTKVDKKVEPKSCDKTHTCPPCPAPELLGGPSVFLFPPKPKDTLMISRTPEVTCVVVDVSHEDPEVKFNWYVDGVEVHNAKTKPREEQYNSTYRVVSVLTVLHQDWLNGKEYKCKVSNKALPAPIEKTISKAKGQPREPQVYTLPPSRDELTKNQVSLTCLVKGFYPSDIAVEWESNGQPENNYKTTPPVLDSDGSFFLYSKLTVDKSRWQQGNVFSCSVMHEALHNHYTQKSLSLSPGK

SEQ ID NO: 46 - protein, 449 aa, artificial sequence
  Heavy Chain with CDR-H3 = Ln4p-65*
QVQLVQSGAEVKKPGASVKVSCKAFGYPFTDYLLHWVRQAPGQGLEWVGWLNPYSGDTNYAQKFQGRVTMTRDTSISTAYMELSRLRSDDTAVYYCARSGLIMDKLDNWGQGTMVTVSSASTKGPSVFPLAPSSKSTSGGTAALGCLVKDYFPEPVTVSWNSGALTSGVHTFPAVLQSSGLYSLSSVVTVPSSSLGTQTYICNVNHKPSNTKVDKKVEPKSCDKTHTCPPCPAPELLGGPSVFLFPPKPKDTLMISRTPEVTCVVVDVSHEDPEVKFNWYVDGVEVHNAKTKPREEQYNSTYRVVSVLTVLHQDWLNGKEYKCKVSNKALPAPIEKTISKAKGQPREPQVYTLPPSRDELTKNQVSLTCLVKGFYPSDIAVEWESNGQPENNYKTTPPVLDSDGSFFLYSKLTVDKSRWQQGNVFSCSVMHEALHNHYTQKSLSLSPGK

SEQ ID NO: 47 - protein, 449 aa, artificial sequence
  Heavy Chain with CDR-H3 = Ln4p-90*
QVQLVQSGAEVKKPGASVKVSCKAFGYPFTDYLLHWVRQAPGQGLEWVGWLNPYSGDTNYAQKFQGRVTMTRDTSISTAYMELSRLRSDDTAVYYCARSGLIIDNLNPWGQGTMVTVSSASTKGPSVFPLAPSSKSTSGGTAALGCLVKDYFPEPVTVSWNSGALTSGVHTFPAVLQSSGLYSLSSVVTVPSSSLGTQTYICNVNHKPSNTKVDKKVEPKSCDKTHTCPPCPAPELLGGPSVFLFPPKPKDTLMISRTPEVTCVVVDVSHEDPEVKFNWYVDGVEVHNAKTKPREEQYNSTYRVVSVLTVLHQDWLNGKEYKCKVSNKALPAPIEKTISKAKGQPREPQVYTLPPSRDELTKNQVSLTCLVKGFYPSDIAVEWESNGQPENNYKTTPPVLDSDGSFFLYSKLTVDKSRWQQGNVFSCSVMHEALHNHYTQKSLSLSPGK

SEQ ID NO: 48 - protein, 449 aa, artificial sequence
  Heavy Chain with CDR-H3 = 3077*
QVQLVQSGAEVKKPGASVKVSCKAFGYPFTDYLLHWVRQAPGQGLEWVGWLNPYSGDTNYAQKFQGRVTMTRDTSISTAYMELSRLRSDDTAVYYCTRSGLIAVYFDYWGQGTMVTVSSASTKGPSVFPLAPSSKSTSGGTAALGCLVKDYFPEPVTVSWNSGALTSGVHTFPAVLQSSGLYSLSSVVTVPSSSLGTQTYICNVNHKPSNTKVDKKVEPKSCDKTHTCPPCPAPELLGGPSVFLFPPKPKDTLMISRTPEVTCVVVDVSHEDPEVKFNWYVDGVEVHNAKTKPREEQYNSTYRVVSVLTVLHQDWLNGKEYKCKVSNKALPAPIEKTISKAKGQPREPQVYTLPPSRDELTKNQVSLTCLVKGFYPSDIAVEWESNGQPENNYKTTPPVLDSDGSFFLYSKLTVDKSRWQQGNVFSCSVMHEALHNHYTQKSLSLSPGK

SEQ ID NO: 49 - protein, 127 aa, human GM-CSF [sequence omitted]

SEQ ID NO: 50 - protein, 127 aa, macaca GM-CSF
APARSPSPGTQPWEHVNAIQEARRLLNLSRDTAAEMNKTVEVVSEMFDLQEPSCLQTRLELYKQGLQGSLTKLKGPLTMMASHYKQHCPPTPETSCATQIITFQSFKENLKDFLLVIPFDCWEPVQE

SEQ ID NO: 51 - protein, 127 aa, gibbon GM-CSF
APSRSPSPSTQPWEHVNAIQEARRLLNLSRDTAAEINETVEVVSEMFDLQEPTCLQTRLELYKQGLRGSLTKLKGPLTMMASHYKQHCPPTPETSCATQIIIFESFKENLKDFLLVIPFDCWEPVQG

SEQ ID NO: 52 - protein, 119 aa, artificial sequence
  VH with CDR-H3 7B1-502
EVQLLESGAEVKKPGASVKVSCKAFGYPFTDYLLHWVRQAPGQGLEWVGWLNPYSGDTNYAQKFQGRVTMTRDTSISTAYMELSRLRSDDTAVYYCTRTTLISVYFDYWGQGTMVTVSS

SEQ ID NO: 53 - protein, 119 aa, artificial sequence
  VH with CDR-H3 3077
EVQLLESGAEVKKPGASVKVSCKAFGYPFTDYLLHWVRQAPGQGLEWVGWLNPYSGDTNYAQKFQGRVTMTRDTSISTAYMELSRLRSDDTAVYYCTRSGLIAVYFDYWGQGTMVTVSS

SEQ ID NO: 54 - protein, 107 aa, artificial sequence
  VL 5-306
ELVMTQSPSSVSASVGDRVTIACRASQNIRNILNWYQQRPGKAPQLLIYAASNLQSGVPSRFSGSGSGTDFTLTINSLQPEDFATYYCQQSYSMPRTFGGGTKVEIK

SEQ ID NO: 55 - protein, 107 aa, artificial sequence
  VL 5-306* V-version
DIQMTQSPSSVSASVGDRVTIACRASQNIRNILNWYQQRPGKAPQLLIYAASNLQSGVPSRFSGSGSGTDFTLTINSLQPEDFATYYCQQSYSMPRTFGGGTKVEIK

SEQ ID NO: 56 - protein, 10 aa, artificial sequence
  CDR-H3 3077
SGLIAVYFDY

SEQ ID NO: 57 - protein, 127 aa, human [sequence omitted]

SEQ ID NO: 58 - protein, 127 aa, Gibbon [sequence omitted]

SEQ ID NO: 59 - protein, 127 aa, rhesus monkey; identical to SEQ ID NO: 50

SEQ ID NO: 60 - protein, 127 aa, cynomolgous monkey; identical to SEQ ID NO: 50